European Patent Application EP 4 692 120 A1, published February 11, 2026. Title: Anti-LAG3 ANTIBODY, PHARMACEUTICAL COMPOSITION, AND USE. Applicant: Akeso Biopharma Co., Ltd. Application WO PCT/CN2024/084453, filed March 28, 2024. The sequence listing filed with the application follows.

SEQUENCE LISTING (25 sequences)

SEQ ID NO: 1 - DNA, 360 bp, synthetic construct
  source 1..360: mol_type = other DNA
caggtgcagctgcagcagtggggagctggactgctgaaacctagcgagacactgagcctgacctgtgctgtgtacggcggatctatcagcgattactactggaactggatcaggcagccccctggaaagggactggaatggatcggagagatcaactacaggggcaccaccaactccaatccctctctgaagagcagggtgacactgagcctcgacacaagcaagaatcagttcagcctgaagctgaggtccgtgaccgctgctgatacagctgtgtactactgtgccttcggctacagcgattacgagtacgattggttcgacccttggggccagggaacactggttacagtgagctcc

SEQ ID NO: 2 - protein, 120 aa, synthetic construct
QVQLQQWGAGLLKPSETLSLTCAVYGGSISDYYWNWIRQPPGKGLEWIGEINYRGTTNSNPSLKSRVTLSLDTSKNQFSLKLRSVTAADTAVYYCAFGYSDYEYDWFDPWGQGTLVTVSS

SEQ ID NO: 3 - DNA, 321 bp, synthetic construct
  source 1..321: mol_type = other DNA
gagatcgttctgacccagagcccagctacactgagcctgtctcctggagagagggctacactgtcctgcagagctagccagaccatcagcagctacctggcttggtaccagcagaagcctggccaagctccaaggctgctgatctacgacgcctctaatagggccaccggcatccctgctagattctctggaagcggcagcggaaccgactttacactgacaatcagctccctggagcccgaggatttcgctgtttactactgtcagcagcgcagcaactggcccatcacattcggacagggcacaaatctggagatcaag

SEQ ID NO: 4 - protein, 107 aa, synthetic construct
EIVLTQSPATLSLSPGERATLSCRASQTISSYLAWYQQKPGQAPRLLIYDASNRATGIPARFSGSGSGTDFTLTISSLEPEDFAVYYCQQRSNWPITFGQGTNLEIK

SEQ ID NO: 5 - DNA, 321 bp, synthetic construct
  source 1..321: mol_type = other DNA
gagatcgttctgacccagagcccagctacactgagcctgtctcctggagagagggctacactgtcctgcagagctagccagaccatcagcagctacctggcttggtaccagcagaagcctggccaagctccaaggctgctgatctacgacggctctaatagggccaccggcatccctgctagattctctggaagcggcagcggaaccgactttacactgacaatcagctccctggagcccgaggatttcgctgtttactactgtcagcagcgcagcaactggcccctcacattcggacagggcacaaatctggagatcaag

SEQ ID NO: 6 - protein, 107 aa, synthetic construct
EIVLTQSPATLSLSPGERATLSCRASQTISSYLAWYQQKPGQAPRLLIYDGSNRATGIPARFSGSGSGTDFTLTISSLEPEDFAVYYCQQRSNWPLTFGQGTNLEIK

SEQ ID NO: 7 - DNA, 321 bp, synthetic construct
  source 1..321: mol_type = other DNA
gagatcgttctgacccagagcccagctacactgagcctgtctcctggagagagggctacactgtcctgcagagctagccagtccatcagcagctacctggcttggtaccagcagaagcctggccaagctccaaggctgctgatctacgacggctctaatagggccaccggcatccctgctagattctctggaagcggcagcggaaccgactttacactgacaatcagctccctggagcccgaggatttcgctgtttactactgtcagcagcgcagcaactggcccatcacattcggacagggcacaaatctggagatcaag

SEQ ID NO: 8 - protein, 107 aa, synthetic construct
EIVLTQSPATLSLSPGERATLSCRASQSISSYLAWYQQKPGQAPRLLIYDGSNRATGIPARFSGSGSGTDFTLTISSLEPEDFAVYYCQQRSNWPITFGQGTNLEIK

SEQ ID NO: 9 - protein, 8 aa, synthetic construct
GGSISDYY

SEQ ID NO: 10 - protein, 7 aa, synthetic construct
INYRGTT

SEQ ID NO: 11 - protein, 14 aa, synthetic construct
AFGYSDYEYDWFDP

SEQ ID NO: 12 - protein, 6 aa, synthetic construct
QTISSY

SEQ ID NO: 13 - skipped

SEQ ID NO: 14 - protein, 9 aa, synthetic construct
QQRSNWPIT

SEQ ID NO: 15 - skipped

SEQ ID NO: 16 - protein, 9 aa, synthetic construct
QQRSNWPLT

SEQ ID NO: 17 - protein, 6 aa, synthetic construct
QSISSY

SEQ ID NO: 18 - protein, 330 aa, synthetic construct [sequence omitted]

SEQ ID NO: 19 - protein, 107 aa, synthetic construct [sequence omitted]

SEQ ID NO: 20 - protein, 327 aa, synthetic construct
ASTKGPSVFPLAPCSRSTSESTAALGCLVKDYFPEPVTVSWNSGALTSGVHTFPAVLQSSGLYSLSSVVTVPSSSLGTKTYTCNVDHKPSNTKVDKRVESKYGPPCPPCPAPEFLGGPSVFLFPPKPKDTLMISRTPEVTCVVVDVSQEDPEVQFNWYVDGVEVHNAKTKPREEQFNSTYRVVSVLTVLHQDWLNGKEYKCKVSNKGLPSSIEKTISKAKGQPREPQVYTLPPSQEEMTKNQVSLTCLVKGFYPSDIAVEWESNGQPENNYKTTPPVLDSDGSFFLYSRLTVDKSRWQEGNVFSCSVMHEALHNHYTQKSLSLSLGK

SEQ ID NO: 21 - protein, 448 aa, synthetic construct
EVQLVESGGGLVQPGGSLRLSCAASGFAFSSYDMSWVRQAPGKGLDWVATISGGGRYTYYPDSVKGRFTISRDNSKNNLYLQMNSLRAEDTALYYCANRYGEAWFAYWGQGTLVTVSSASTKGPSVFPLAPSSKSTSGGTAALGCLVKDYFPEPVTVSWNSGALTSGVHTFPAVLQSSGLYSLSSVVTVPSSSLGTQTYICNVNHKPSNTKVDKKVEPKSCDKTHTCPPCPAPEAAGAPSVFLFPPKPKDTLMISRTPEVTCVVVDVSHEDPEVKFNWYVDGVEVHNAKTKPREEQYNSTYRVVSVLTVLHQDWLNGKEYKCKVSNKALPAPIEKTISKAKGQPREPQVYTLPPSRDELTKNQVSLTCLVKGFYPSDIAVEWESNGQPENNYKTTPPVLDSDGSFFLYSKLTVDKSRWQQGNVFSCSVMHEALHNHYTQKSLSLSPGK

SEQ ID NO: 22 - protein, 214 aa, synthetic construct
DIQMTQSPSSMSASVGDRVTFTCRASQDINTYLSWFQQKPGKSPKTLIYRANRLVSGVPSRFSGSGSGQDYTLTISSLQPEDMATYYCLQYDEFPLTFGAGTKLELKRTVAAPSVFIFPPSDEQLKSGTASVVCLLNNFYPREAKVQWKVDNALQSGNSQESVTEQDSKDSTYSLSSTLTLSKADYEKHKVYACEVTHQGLSSPVTKSFNRGEC

SEQ ID NO: 23 - protein, 447 aa, synthetic construct
QVQLQQWGAGLLKPSETLSLTCAVYGGSFSDYYWNWIRQPPGKGLEWIGEINHRGSTNSNPSLKSRVTLSLDTSKNQFSLKLRSVTAADTAVYYCAFGYSDYEYNWFDPWGQGTLVTVSSASTKGPSVFPLAPCSRSTSESTAALGCLVKDYFPEPVTVSWNSGALTSGVHTFPAVLQSSGLYSLSSVVTVPSSSLGTKTYTCNVDHKPSNTKVDKRVESKYGPPCPPCPAPEFLGGPSVFLFPPKPKDTLMISRTPEVTCVVVDVSQEDPEVQFNWYVDGVEVHNAKTKPREEQFNSTYRVVSVLTVLHQDWLNGKEYKCKVSNKGLPSSIEKTISKAKGQPREPQVYTLPPSQEEMTKNQVSLTCLVKGFYPSDIAVEWESNGQPENNYKTTPPVLDSDGSFFLYSRLTVDKSRWQEGNVFSCSVMHEALHNHYTQKSLSLSLGK

SEQ ID NO: 24 - protein, 214 aa, synthetic construct
EIVLTQSPATLSLSPGERATLSCRASQSISSYLAWYQQKPGQAPRLLIYDASNRATGIPARFSGSGSGTDFTLTISSLEPEDFAVYYCQQRSNWPLTFGQGTNLEIKRTVAAPSVFIFPPSDEQLKSGTASVVCLLNNFYPREAKVQWKVDNALQSGNSQESVTEQDSKDSTYSLSSTLTLSKADYEKHKVYACEVTHQGLSSPVTKSFNRGEC

SEQ ID NO: 25 - protein, 669 aa, synthetic construct
LQPGAEVPVVWAQEGAPAQLPCSPTIPLQDLSLLRRAGVTWQHQPDSGPPAAAPGHPLAPGPHPAAPSSWGPRPRRYTVLSVGPGGLRSGRLPLQPRVQLDERGRQRGDFSLWLRPARRADAGEYRAAVHLRDRALSCRLRLRLGQASMTASPPGSLRASDWVILNCSFSRPDRPASVHWFRNRGQGRVPVRESPHHHLAESFLFLPQVSPMDSGPWGCILTYRDGFNVSIMYNLTVLGLEPPTPLTVYAGAGSRVGLPCRLPAGVGTRSFLTAKWTPPGGGPDLLVTGDNGDFTLRLEDVSQAQAGTYTCHIHLQEQQLNATVTLAIITVTPKSFGSPGSLGKLLCEVTPVSGQERFVWSSLDTPSQRSFSGPWLEAQEAQLLSQPWQCQLYQGERLLGAAVYFTELSSPGAQRSGRAPGALPAGHLKLENLYFQGPRGPTIKPCPPCKCPAPNLLGGPSVFIFPPKIKDVLMISLSPIVTCVVVDVSEDDPDVQISWFVNNVEVHTAQTQTHREDYNSTLRVVSALPIQHQDWMSGKEFKCKVNNKDLPAPIERTISKPKGSVRAPQVYVLPPPEEEMTKKQVTLTCMVTDFMPEDIYVEWTNNGKTELNYKNTEPVLDSDGSYFMYSKLRVEKKNWVERNSYSCSVVHEGLHNHHTTKSFSRTPGK